European Patent Specification EP 3 768 079 B1, published April 29, 2026. Title: TRANSGENIC CHICKEN THAT PRODUCES HUMAN ANTIBODIES. Applicant: Crystal Bioscience Inc. Leighton, Philip  A Harriman, William D. The sequence listing filed with the application follows.

SEQUENCE LISTING (58 sequences)

SEQ ID NO: 1 - DNA, 23 bp, Artificial sequence
  synthetic sequence
caccagtcggctccgcaaccatg

SEQ ID NO: 2 - DNA, 18 bp, Artificial sequence
  synthetic sequence
gggcgatgtggggctcgc

SEQ ID NO: 3 - protein, 19 aa, Artificial sequence
  synthetic sequence
MSPLVSSLLLLAALPGLMA

SEQ ID NO: 4 - protein, 19 aa, Artificial sequence
  synthetic sequence
MEFGLSWIFLVAILKGVQC

SEQ ID NO: 5 - protein, 19 aa, Artificial sequence
  synthetic sequence
MEFGLSWLFLVAKIKGVQC

SEQ ID NO: 6 - protein, 118 aa, Artificial sequence
  synthetic sequence
DVQLVESGGGVVRPGESLRLSCAASGFTFTNYDMSWVRQAPGEGLEWVSAISGSGDTTYYADSVKGRFTISRDNSKNTLYLRLFSLRAEDTAIYYCAKGTWNTFFDYWGLGTLVTVSS

SEQ ID NO: 7 - protein, 118 aa, Artificial sequence
  synthetic sequence
EVQLVESGGGLVQPGGSLRLSCAVSGFPFSSYAMSWVRQAPGEGLEWVSASSGSGAITYYADSVKGRFTISRDNSKNTLYLRLFSLRAEDTAIYYCAKDMVPYREGGNSGYYYGMDVD

SEQ ID NO: 8 - protein, 118 aa, Artificial sequence
  synthetic sequence
DVQLVESGGGVVRPGESLRLSCAASGFTFSSSARSWVRQAPGKGLEWVSAISGSGGSTFYADSVKGRFTISRDNSKNTLYLRLFSLRAEDTAIYYCAKAWELLHIQPDAAPGFSGAHS

SEQ ID NO: 9 - protein, 118 aa, Artificial sequence
  synthetic sequence
EVQLVESGGGLVQPGGSLRLSCAASGFSFSSYAMSWVRQAPGEGLEWVSIISVSGTSTYYADSVKGRFTISRDNSKNTLYLRLFSLRAEDTAIYYCARDRGGIAAQDTHGVHVSRAAL

SEQ ID NO: 10 - protein, 118 aa, Artificial sequence
  synthetic sequence
DVQLVESGGGVVRPGESLRLSCAASGFTFSNYGMTWVRQPPGKGLEWVSGIRGSGGGAYYADSVRGRFTVSRDNSKNTLYLQMNSLRAEDTAVYYCAKDSTVSWYRALFQHTPGFMES

SEQ ID NO: 11 - protein, 118 aa, Artificial sequence
  synthetic sequence
EVQLVESGGGLVQPGGSLRLSCAASGFTFTSYAMSWVRQAPGEGLEWVSSISGNGGSTYYADSVKGRFTISRDNSKNTLYLRLFSLRAEDTAIYYCAKDLGYYYDSSGDYGGSRGMDV

SEQ ID NO: 12 - protein, 118 aa, Artificial sequence
  synthetic sequence
DVQLVESGGGVVRPGESLRLSCAASGFTFSSYGMSWVRQAPGEGLEWVSGISASGNSAYYADSVKGRFTISRDNSKNTLYLRLFSLRAEDTAIYYCAEDSYNTGWTEYFQHIDGKGMR

SEQ ID NO: 13 - protein, 118 aa, Artificial sequence
  synthetic sequence
DVQLVESGGGVVRPGESLRLSCAASGFTFSSYDMSWVRQAPGEGLEWVSGISGRGGSTYYADSVKGRFTISRDNSKNTLYLRLFSLRAEDTAIYYCAKPEGGRGAAAGPFDAFDISPG

SEQ ID NO: 14 - protein, 118 aa, Artificial sequence
  synthetic sequence
DVQLVESGGGVVRPGESLRLSCAASGFTFDIYAMSWVRQAPGKGLEWVSAISGSAYSTYYADSVKGRFTISRDSSKNTLYLQMNSLRAEDTAVYYCAKDGIAAGHTRARGSAYPGEMD

SEQ ID NO: 15 - protein, 118 aa, Artificial sequence
  synthetic sequence
DVQLVESGGGVVRPGESLRLSCAASGFTFSNFAMTWVRQAPGKGPEWVSAISHSGGSTYSADSVKGRFTISRDNSKNTLYLRLFSLRAEDTAIYYCAKRDRRSSIAARLLGYYYYYGM

SEQ ID NO: 16 - protein, 118 aa, Artificial sequence
  synthetic sequence
DVQLVESGGGVVRPGESLRLSCAASGFTFSSHAMSWVRQAPGEGLEWVSAISGNGVSAYYADSVKGRFTISRDNSKNTLYLRLFSLRAEDTAIYYCAKDPFGYSNYGFDYFASVSPGF

SEQ ID NO: 17 - protein, 118 aa, Artificial sequence
  synthetic sequence
DVQLVESGGGVVRPGESLRLSCAASGFTFSTYAMSWVRQAPGEGLEWVSRISGSGGSTDYAESVKGRFTISRDNSKNTLYLRLFSLRAEDTAIYYCARSKEDYDILTGYNLQYYYYGM

SEQ ID NO: 18 - protein, 118 aa, Artificial sequence
  synthetic sequence
DVQLVESGGGVVRPGESLRLSCAASGFTFSSYAVSWVRQAPGKGLEWVSAISGSADSTYYADSVKGRFTISRDNSKSTLYLQMNSLRAEDTAVYYCAKSGRFGDLWEVYYYGLDVAYR

SEQ ID NO: 19 - protein, 118 aa, Artificial sequence
  synthetic sequence
DVQLVESGGGVVRPGESLRLSCAASGFSFSSYAMNWVRQAPGEGLEWVSGISGRGGSTYYADSVKGRFTISRDNSKNTLYLRLFSLRAEDTAIYYCARDFRYYDAINNYGILVTWTAR

SEQ ID NO: 20 - protein, 118 aa, Artificial sequence
  synthetic sequence
DVQLVESGGGVVRPGESLRLSCAASGFTFRSYAMNWVRQAPGEGLEWVSLISGSGESIYYADSVKGRFTISRDNSKNTLYLQMNSLRAEDTAVYYCANREQLWFSSGETYYYYYGMDV

SEQ ID NO: 21 - protein, 118 aa, Artificial sequence
  synthetic sequence
DVQLVESGGGVVRPGESLRLSCAASGFTFSNYAMTWVRQAPGEGLEWVSVISSSGDTTYYADSVKGRFTISRDNSKNTLYLRLFSLRAEDTAIYYCAKDRWWGTDSDAGVGQHSGLIV

SEQ ID NO: 22 - protein, 118 aa, Artificial sequence
  synthetic sequence
EVQLLDSGGGLVQPGGSLTLSCAASGFTFSNYAMGWVRQAPGEGLEWVSGISASGGSTYYADSVKGRFTISRDNSKNTLYLRLFSLRAEDTAIYYCAKENNRHGGVSTFGGVLTSPHG

SEQ ID NO: 23 - protein, 118 aa, Artificial sequence
  synthetic sequence
DVQLVESGGGVVRPGESLRLSCAASGFTFSSYVMSWVRQAPGEGLEWVSDIRGSGDSTYYSDSVKGRFTISRDNSKNTLYLRLFSLRAEDTAIYYCAKAAAHYYDILTGYFPSYYYYG

SEQ ID NO: 24 - protein, 118 aa, Artificial sequence
  synthetic sequence
DVQLVESGGGVVRPGESLRLSCAASGFTFSIYAMSWVRQAPGEGLEWVSVIIGSGDRIHYADSVKGRFTISRDSSNNTLYLQMNSLRAEDTAVYYCAKISGDIVVVPAAFHDVAPGLN

SEQ ID NO: 25 - protein, 118 aa, Artificial sequence
  synthetic sequence
EVQLVESGGGLVQPGGSLRLSCTASGFTFRNYAMPWVRQAPGEGLEWVSTLSDNGGSTYYADSVKGRFTISRDNSKNTLYLRLFSLRAEDTAIYYCAKGASRNSLLPYNPGFGGVIHS

SEQ ID NO: 26 - protein, 118 aa, Artificial sequence
  synthetic sequence
DVQLVESGGGVVRPGESLRLSCAASGFTFSSDAMSWVRQAPGEGLEWVSSISGSGLNTDYADSVKGRFTISRDNSKNTLYLRLFSLRAEDTAIYYCAKVGWELPYGVSPGFGGLAHGP

SEQ ID NO: 27 - protein, 124 aa, Artificial sequence
  synthetic sequence
EVQLLESGGGLVQPGGSLRLSCAASGFTFSSYAMSWVRQAPGKGLEWVSAISGSGGSTYYADSVKGRFTISRDNSKNTLYLQMNSLRAEDTAVYYCAKEYNWNDYYYYYGMDVWGQGTTVTVSS

SEQ ID NO: 28 - protein, 115 aa, Artificial sequence
  synthetic sequence
EVQLLESGGGLVQPGGSLRLSCAASGFTFSSYWMSWVRQAPGKGLEWVSAIKQDGSEKYYADSVKGRFTISRDNSKNTLYLQMNSLRAEDTAVYYCAKNPGFGGVIHSPHGEIRA

SEQ ID NO: 29 - protein, 115 aa, Artificial sequence
  synthetic sequence
EVQLLESGGGLVQPGGSLRLSCAASGFTFDDYAMSWVRQAPGKGLEWVSAISWNSGSIYYADSVKGRFTISRDNSKNTLYLQMNSLRAEDTAVYYCAKDVAPGLNGGLRDPIPGE

SEQ ID NO: 30 - protein, 115 aa, Artificial sequence
  synthetic sequence
EVQLLESGGGLVQPGGSLRLSCAASGFTFSDYYMSWVRQAPGKGLEWVSAISSSGSTIYYADSVKGRFTISRDNSKNTLYLQMNSLRAEDTAVYYCAKARTGLTGTRVHLHLGRL

SEQ ID NO: 31 - protein, 115 aa, Artificial sequence
  synthetic sequence
EVQLLESGGGLVQPGGSLRLSCAASGFTFSSYDMSWVRQAPGKGLEWVSAIGTAGDTYYYADSVKGRFTISRDNSKNTLYLQMNSLRAEDTAVYYCAKGGSHRHHRVASSSASGK

SEQ ID NO: 32 - protein, 116 aa, Artificial sequence
  synthetic sequence
EVQLLESGGGLVQPGGSLRLSCAASGFTFSNAWMSWVRQAPGKGLEWVSAIKSKTDGGTTYYADSVKGRFTISRDNSKNTLYLQMNSLRAEDTAVYYCAKGMEREVMTIKPECPTP

SEQ ID NO: 33 - protein, 115 aa, Artificial sequence
  synthetic sequence
EVQLLESGGGLVQPGGSLRLSCAASGFTFDDYGMSWVRQAPGKGLEWVSAINWNGGSTYYADSVKGRFTISRDNSKNTLYLQMNSLRAEDTAVYYCAKPPTPTCPTPRPPLTEPM

SEQ ID NO: 34 - protein, 115 aa, Artificial sequence
  synthetic sequence
EVQLLESGGGLVQPGGSLRLSCAASGFTFSSYSMSWVRQAPGKGLEWVSAISSSSSYIYYADSVKGRFTISRDNSKNTLYLQMNSLRAEDTAVYYCAKILVTWTARGHDFICIWE

SEQ ID NO: 35 - protein, 115 aa, Artificial sequence
  synthetic sequence
EVQLLESGGGLVQPGGSLRLSCAASGFTFSSYAMSWVRQAPGKGLEWVSAISYDGSNKYYADSVKGRFTISRDNSKNTLYLQMNSLRAEDTAVYYCAKRAPISPRGLWAPLNPGA

SEQ ID NO: 36 - protein, 114 aa, Artificial sequence
  synthetic sequence
EVQLLESGGGLVQPGGSLRLSCAASGFTVSSNYMSWVRQAPGKGLEWVSAIYSGGSTYYADSVKGRFTISRDNSKNTLYLQMNSLRAEDTAVYYCAKRALISQPGWSVTPLSAE

SEQ ID NO: 37 - protein, 113 aa, Artificial sequence
  synthetic sequence
EVQLLESGGGLVQPGGSLRLSCAASGFTFSSYAMSWVRQAPGKGLEWVSAISSNGGSTYYADSVKGRFTISRDNSKNTLYLQMNSLRAEDTAVYYCAKRCTTRVPLPSISPGA

SEQ ID NO: 38 - protein, 117 aa, Artificial sequence
  synthetic sequence
EVQLLESGGGLVQPGGSLRLSCAASGFTFSDHYMSWVRQAPGKGLEWVSATRNKANSYTTYYADSVKGRFTISRDNSKNTLYLQMNSLRAEDTAVYYCAKSPGLGSLSLPRNPGPTL

SEQ ID NO: 39 - protein, 116 aa, Artificial sequence
  synthetic sequence
EVQLLESGGGLVQPGGSLRLSCAASGFTFSGSAMSWVRQAPGKGLEWVSAIRSKANSYATYYADSVKGRFTISRDNSKNTLYLQMNSLRAEDTAVYYCAKQGGPSKGRTRIPLPSM

SEQ ID NO: 40 - protein, 114 aa, Artificial sequence
  synthetic sequence
EVQLLESGGGLVQPGGSLRLSCAASGFTFSSYWMSWVRQAPGKGLEWVSAINSDGSSTYYADSVKGRFTISRDNSKNTLYLQMNSLRAEDTAVYYCAKGSMTECPPMPRWTEQR

SEQ ID NO: 41 - DNA, 122 bp, Artificial sequence
  synthetic sequence
gtggataacgataattagaaggggacaaattaatgagaaaacacgactccgggcctagacggccattaaatcattaatcaacccgacgggcgcccaattaatcataaagttattaagcaatt

SEQ ID NO: 42 - DNA, 122 bp, Artificial sequence
  synthetic sequence
aattgcttaataactttatgattaattgggcgcccgtcgggttgattaatgatttaatggccgtctaggcccggagtcgtgttttctcattaatttgtccccttctaattatcgttatccac

SEQ ID NO: 43 - DNA, 20 bp, Artificial sequence
  synthetic sequence
aaatcattaatcaacccgac

SEQ ID NO: 44 - DNA, 20 bp, Artificial sequence
  synthetic sequence
aacacgactccgggcctaga

SEQ ID NO: 45 - DNA, 20 bp, Artificial sequence
  synthetic sequence
tgattaattgggcgcccgtc

SEQ ID NO: 46 - DNA, 20 bp, Artificial sequence
  synthetic sequence
atttaatggccgtctaggcc

SEQ ID NO: 47 - DNA, 19 bp, Artificial sequence
  synthetic sequence
aagttcgagggcgacaccc

SEQ ID NO: 48 - DNA, 25 bp, Artificial sequence
  synthetic sequence
gcccctaataagtggtttaattatg

SEQ ID NO: 49 - DNA, 20 bp, Artificial sequence
  synthetic sequence
tctgcgctgagttctttgat

SEQ ID NO: 50 - DNA, 20 bp, Artificial sequence
  synthetic sequence
aagtcgaggctgacgagaaa

SEQ ID NO: 51 - DNA, 20 bp, Artificial sequence
  synthetic sequence
cttttccccaccaaatttca

SEQ ID NO: 52 - DNA, 24 bp, Artificial sequence
  synthetic sequence
tggtttggttgatggaagaatgta

SEQ ID NO: 53 - DNA, 23 bp, Artificial sequence
  synthetic sequence
atacgatgttccagattacgctt

SEQ ID NO: 54 - DNA, 22 bp, Artificial sequence
  synthetic sequence
gctgaactagaatgcatcaagc

SEQ ID NO: 55 - DNA, 20 bp, Artificial sequence
  synthetic sequence
acaaacctttgccgcatcca

SEQ ID NO: 56 - DNA, 24 bp, Artificial sequence
  synthetic sequence
gatggggggtggcaatggaatgat

SEQ ID NO: 57 - DNA, 22 bp, Artificial sequence
  synthetic sequence
agctgtgctcgacgttgtcact

SEQ ID NO: 58 - DNA, 20 bp, Artificial sequence
  synthetic sequence
gcccaaaatggccccaaaac